European Patent Application EP 4 556 569 A1, published May 21, 2025. Title: METHOD FOR AGAROSE LIQUEFACTION AND NA4/NA6 PRODUCTION USING THERMOSTABLE GH6B β-AGARASE DERIVED FROM A NOVEL AGAR-DEGRADING BACTERIUM. Applicant: 경북대학교 산학협력단. The sequence listing filed with the application follows.

SEQUENCE LISTING (13 sequences)

SEQ ID NO: 1 - protein, 597 aa, Cellvibrio sp. KY-GH-1
MKKITSCIAAALLLSAPLASFAADWDSVPIPAAAGTGKTWQLQSISDEFNYTASPTVKPAEFNTRWNPSFINSWTGPGDSEFNAGHSYTSGGSLALQSSAKAGTNKIYTGIISSKETFTYPLYLEARVKHTGNTLANAVWMLSADSTQEIDAMESYGSDRAGQEWFDQRMHVSHHVFIRSPFQDYQPKDEGSWVVNPAGGTWRGAMHVYGVHWKDPWNLDYYIDGVKVRTVSGPAMIDPYNFTNGTGINKPLHIIIDVEHQDWRDVRPTAAELADTSKSIMFVDWIRVYKPVTSSATSSSNSVSSSSSSLSNSSSSSATTVIDFANYFDTGKSTASVAGDTYVGFNKSGSGNINYNTAGDWADYLVTLPSDGQYKIEVTTASPMTSGIGAKLSVDGIYVSTTSLAATGGWELYSASTLANNLSIGAGTHTVRIESTGTSAWQWNGDEIRVTKVGSAPVGSPTTPAPVAMIIQAESFSATGGVYDGFKTYSVNGVSAINYNQRGDWADYAVNVAADGSYTFNAYVSSPMSGAALEVSVDGVKVLTQAVPNNGSWDSFQKVSSASKIALTKGAHTIRVTSAGTTSSTWEWNADKFELIP

SEQ ID NO: 2 - protein, 477 aa, Cellvibrio sp. KY-GH-1
MKKHISCCIALMLTSVASLAADWDAYPVPASAGAGKVWQLQSQSDEFNYNFSATAAAATFGGKWTNFYHNTWEGPGPTRWMRENTSVSGGQLQIKATRVAGETKTYDVDLNLDGVNEQFTSPATRAGCITSTTRVKYPVFIEARVKIANAVMASDVWMLSPDDTEEIDILEAYGGKAARNDWFAQRLHLSHHLFIRNPFTDYQPRDASTWYAGAGVTYWADNWVRIGVNWVSPTRLEYYVNGQLVKVMDKLNTVNGIDGIDPWNITGGKGITKEMDIIINMEDQNWNAAQGRQPTDAEITNASNHTFKVDWIRVYKPVTATTSSSSSNGSAASSASSNTVQLIDFANYFDTGKVTASVSGDNYIGFNKSGGGNINYNTVGDWGDYLVTLPNDGKYKFEIITASPMTSGLGAKLIIDGIYVGTISVGSTGGWEVYSAFALANSISIGAGTHTVRIESTGSSSWQWNGDQIRITRVGSL

SEQ ID NO: 3 - protein, 590 aa, Cellvibrio sp. KY-GH-1
MQLIDNKEENIKMKKLTQRKLFYILTLTLFSTSIFAQPTPPAGKMWQKQSNLSDDFNSGFDTSKWQKPLWNYGEPVNMVAENSGVSNGNLWIKGTLGTGARWFNGSRVMSNAQIKYPYYTEARIKSANISAYSTFWLNNGDINNRDEIDIIENNPNPSCNCQPNFPWQMNSQYFHVVNGDTQRAHGNFDNRNLPDGAPGKGVRWNEAYFTFGVWQKDARNIQFYLNGYPAGSVVSARDFTRDMNIIWDLWTADFSWLGGLAVQSQLNDVSMNTMYVDWINTYKLVDGVASSSSSSSAQSSSSANSSVASGATQTIDFANYFDTGKATSAVAGDTIIGFNKSGGGNINYNSVGDWGDYLVTLPTDGQYKIEIVTASPMTSGIGAKLSIDGIAVGTITLGTTGDWETYTTTTLVNNLSIGAGTHTLRIESTGTSAWQWNGDVIRVTKVGSDPIGSPVTPTPVSMTLQAENFAATGGVYDGFKIYTVNGVSAVNYNQRGDWANYTVNVAADGNYSFNAYVSSPMTGAALEVTVDGVKVLTQAVPNNGSWDNFQKISSSNKIALTKGTHTIRVASAGTTASTWEWNADKFELVP

SEQ ID NO: 4 - protein, 998 aa, Cellvibrio sp. KY-GH-1
MRIRSPWSATEAIVRDNTPAAQSFPLSDLSNKAGWRFVPTASDEFNQATLDVLKSPSDSTGKWVTNNHTWGGREPAPFLPKNVRQESGLLKLSLKQKVESQIYGFLNANFMNGWSAATAMNATPVRYGYFEVRSKVGVGSSAFWLYSKSMEDVRYIKGERVFTKALVDHNLEIDVYEQAGRRPEWAPYYNMNTWVFEYQGDDHRIFSKKASGQSCGREGWQGGDDLLPHAAGLQNGGHWKADIDFAADFHVYGLYWGPDELRWYVDGKLIRSMKNRYHHTPLYILLDTETMPDWFGLPTPAELQHDHEIDYVRVWTTDALENHNGKGWRAIQADGNARYSMRVAARDGDGHQNGKGANQPLEYLQQHSKPFGTVESYIGSATSGTQNPVKATAVNFKTTDLLVLSERRLSPYRAAADNIRYYYAHYGHVIDAIITPSNATNKNIKWVSDNPAIATVTASGVIVPAQTYDAETGSLTHIASGEVTLTGTHADLPGNVFTLRVKLVEVGSENSITLANFSTTGRNATVAEGYAASAVGWGTKGFPSAITDNTRGEFGSYQIDFGSGGKFSFMLSAGTPIQTGTGVKVFIDDEEVLSENLNNISGDWDAHFENWFPTTFTVSPGKHWVKIMSAGASEWQWFGHSAQFLQLLDGTNSPSSSAASASTMSSRSSVAQSSVAASSVPTSSAAPSSVAKSSIAPSSAVNSSVASSIGGIGAKVIVQAENFIATGGTYQGFQKYTTANGIGAINYNQRGDWADYSFTIGSAGTYTINAFLGTTLADSAIELFIDNVSVGKKTVLNNNNWDAFVPLTLNTGVQLSAGTHTLRVVSAGTTASTWEWNADRIEFTQIAATSSSRSSAASSSSATPTPIVVQAESYTTTGGAYQGLQKYTTATGVAAVNYNQRGDWADYTINVTATGNYRINAYLGTTQVGGAIEILVDGISVAKKTVPNNNNWDVFAALEVSNSVRLTQGMHNVRIISAGATASTWEWNADRIEFVPVN

SEQ ID NO: 5 - DNA, 29 bp, synthetic construct
  source 1..29: mol_type = other DNA
gcggcatatgaaaaaaatcacttcatgta

SEQ ID NO: 6 - DNA, 31 bp, synthetic construct
  source 1..31: mol_type = other DNA
gcggcatatgcagttaatagataataaagag

SEQ ID NO: 7 - DNA, 27 bp, synthetic construct
  source 1..27: mol_type = other DNA
gcggcatatgcgtattcgctcaccttg

SEQ ID NO: 8 - DNA, 28 bp, synthetic construct
  source 1..28: mol_type = other DNA
cgcatatggccgattgggattcagttcc

SEQ ID NO: 9 - DNA, 31 bp, synthetic construct
  source 1..31: mol_type = other DNA
cgggatccatgaaaaagcatatttcatgctg

SEQ ID NO: 10 - DNA, 29 bp, synthetic construct
  source 1..29: mol_type = other DNA
ctaactcgaggggtatcaattcaaacttg

SEQ ID NO: 11 - DNA, 32 bp, synthetic construct
  source 1..32: mol_type = other DNA
cgcgctcgaggggtactaattcaaatttatcc

SEQ ID NO: 12 - DNA, 32 bp, synthetic construct
  source 1..32: mol_type = other DNA
cgcgctcgagatttactggcacaaactcaatg

SEQ ID NO: 13 - DNA, 28 bp, synthetic construct
  source 1..28: mol_type = other DNA
cgaagcttgagtgagccaactcgagtaa